European Patent Application EP 4 420 683 A1, published August 28, 2024. Title: ANTI-CD37 ANTIBODY-DRUG CONJUGATE. Applicant: Daiichi Sankyo Company, Limited. Application EP 22883530.2, filed October 17, 2022. The sequence listing filed with the application follows.

SEQUENCE LISTING (24 sequences)

SEQ ID NO: 1 - DNA, 702 bp, synthetic construct
  misc_feature 1..702: note = nucleotide sequence coding hmAb-L11 light chain
  source 1..702: mol_type = other DNA
  CDS 1..>702: protein_id = 2; translation = MVLQTQVFISLLLWISGAYGDIQMTQSPSSLSASVGDRVTITCKASQDVSTAVDWYQQKPGKAPKLLINWASTRHTGVPSRFSGSGSGTDFTLTISSLQPEDFATYYCRQHYSTPFTFGQGTKVEIKRTVAAPSVFIFPPSDEQLKSGTASVVCLLNNFYPREAKVQWKVDNALQSGNSQESVTEQDSKDSTYSLSSTLTLSKADYEKHKVYACEVTHQGLSSPVTKSFNRGEC
atggtgctgcagacccaggtgttcatctccctgctgctgtggatctccggcgcgtacggcgatatccagatgacacagagccctagcagcctgtctgccagcgtgggagacagagtgaccatcacatgcaaggccagccaggatgtgtccaccgccgtggattggtatcagcagaagcctggcaaggcccctaagctgctgatcaactgggccagcacaagacacacaggcgtgcccagcagattttctggcagcggctctggcaccgacttcaccctgaccatatctagcctgcagcctgaggacttcgccacctactactgcagacagcactacagcacccctttcacctttggccagggcaccaaggtggaaatcaagcgtacggtggccgccccctccgtgttcatcttccccccctccgacgagcagctgaagtccggcaccgcctccgtggtgtgcctgctgaataacttctaccccagagaggccaaggtgcagtggaaggtggacaacgccctgcagtccgggaactcccaggagagcgtgaccgagcaggacagcaaggacagcacctacagcctgagcagcaccctgaccctgagcaaagccgactacgagaagcacaaggtgtacgcctgcgaggtgacccaccagggcctgagctcccccgtcaccaagagcttcaacaggggggagtgt

SEQ ID NO: 2 - protein, 234 aa, synthetic construct
  REGION 1..234: note = Synthetic Construct
MVLQTQVFISLLLWISGAYGDIQMTQSPSSLSASVGDRVTITCKASQDVSTAVDWYQQKPGKAPKLLINWASTRHTGVPSRFSGSGSGTDFTLTISSLQPEDFATYYCRQHYSTPFTFGQGTKVEIKRTVAAPSVFIFPPSDEQLKSGTASVVCLLNNFYPREAKVQWKVDNALQSGNSQESVTEQDSKDSTYSLSSTLTLSKADYEKHKVYACEVTHQGLSSPVTKSFNRGEC

SEQ ID NO: 3 - DNA, 1404 bp, synthetic construct
  misc_feature 1..1404: note = nucleotide sequence coding hmAb-H11 heavy chain
  source 1..1404: mol_type = other DNA
  CDS 1..>1404: protein_id = 4; translation = MKHLWFFLLLVAAPRWVLSEVQLVQSGAEVKKPGASVKVSCKASGYSFTDYNMYWVRQAPGQSLEWMGYIDPYNGDTTYNQKFQGRVTITADTSTSTAYMELSSLRSEDTAVYYCARSPYGHYAMDYWGQGTLVTVSSASTKGPSVFPLAPSSKSTSGGTAALGCLVKDYFPEPVTVSWNSGALTSGVHTFPAVLQSSGLYSLSSVVTVPSSSLGTQTYICNVNHKPSNTKVDKKVEPKSCDKTHTCPPCPAPELLGGPSVFLFPPKPKDTLMISRTPEVTCVVVDVSHEDPEVKFNWYVDGVEVHNAKTKPREEQYNSTYRVVSVLTVLHQDWLNGKEYKCKVSNKALPAPIEKTISKAKGQPREPQVYTLPPSREEMTKNQVSLTCLVKGFYPSDIAVEWESNGQPENNYKTTPPVLDSDGSFFLYSKLTVDKSRWQQGNVFSCSVMHEALHNHYTQKSLSLSPGK
atgaaacacctgtggttcttcctcctgctggtggcagctcccagatgggtgctgagcgaagttcagctggttcagtctggcgccgaagtgaagaaacctggcgcctctgtgaaggtgtcctgcaaggccagcggctacagcttcaccgactacaacatgtactgggtccgacaggcccctggccagtctcttgagtggatgggctacatcgacccctacaacggcgacaccacctacaaccagaaattccagggcagagtgaccatcaccgccgacacctctacaagcaccgcctacatggaactgagcagcctgagaagcgaggacaccgccgtgtactactgcgccagatctccttacggccactacgccatggattactggggccagggaaccctggtcacagttagctcagcctccaccaagggcccaagcgtcttccccctggcaccctcctccaagagcacctctggcggcacagccgccctgggctgcctggtcaaggactacttccccgaacccgtgaccgtgagctggaactcaggcgccctgaccagcggcgtgcacaccttccccgctgtcctgcagtcctcaggactctactccctcagcagcgtggtgaccgtgccctccagcagcttgggcacccagacctacatctgcaacgtgaatcacaagcccagcaacaccaaggtggacaagaaggttgagcccaaatcttgtgacaaaactcacacatgcccaccctgcccagcacctgaactcctggggggaccctcagtcttcctcttccccccaaaacccaaggacaccctcatgatctcccggacccctgaggtcacatgcgtggtggtggacgtgagccacgaagaccctgaggtcaagttcaactggtacgtggacggcgtggaggtgcataatgccaagacaaagccccgggaggagcagtacaacagcacgtaccgggtggtcagcgtcctcaccgtcctgcaccaggactggctgaatggcaaggagtacaagtgcaaggtctccaacaaagccctcccagcccccatcgagaaaaccatctccaaagccaaaggccagccccgggaaccacaggtgtacaccctgcccccatcccgggaggagatgaccaagaaccaggtcagcctgacctgcctggtcaaaggcttctatcccagcgacatcgccgtggagtgggagagcaatggccagcccgagaacaactacaagaccacccctcccgtgctggactccgacggctccttcttcctctacagcaagctcaccgtggacaagagcaggtggcagcagggcaacgtcttctcatgctccgtgatgcatgaggctctgcacaaccactacacccagaagagcctctccctgtctcccggcaaa

SEQ ID NO: 4 - protein, 468 aa, synthetic construct
  REGION 1..468: note = Synthetic Construct
MKHLWFFLLLVAAPRWVLSEVQLVQSGAEVKKPGASVKVSCKASGYSFTDYNMYWVRQAPGQSLEWMGYIDPYNGDTTYNQKFQGRVTITADTSTSTAYMELSSLRSEDTAVYYCARSPYGHYAMDYWGQGTLVTVSSASTKGPSVFPLAPSSKSTSGGTAALGCLVKDYFPEPVTVSWNSGALTSGVHTFPAVLQSSGLYSLSSVVTVPSSSLGTQTYICNVNHKPSNTKVDKKVEPKSCDKTHTCPPCPAPELLGGPSVFLFPPKPKDTLMISRTPEVTCVVVDVSHEDPEVKFNWYVDGVEVHNAKTKPREEQYNSTYRVVSVLTVLHQDWLNGKEYKCKVSNKALPAPIEKTISKAKGQPREPQVYTLPPSREEMTKNQVSLTCLVKGFYPSDIAVEWESNGQPENNYKTTPPVLDSDGSFFLYSKLTVDKSRWQQGNVFSCSVMHEALHNHYTQKSLSLSPGK

SEQ ID NO: 5 - DNA, 1404 bp, synthetic construct
  misc_feature 1..1404: note = nucleotide sequence coding hmAb-H541 heavy chain
  source 1..1404: mol_type = other DNA
  CDS 1..>1404: protein_id = 6; translation = MKHLWFFLLLVAAPRWVLSEVQLVQSGAEVKKPGASVKVSCKASGYSFTDYNMYWVRQAPGQSLEWMGYIDPYNGDTTYNQKFQGRVTMTRDTSISTAYMELSRLRSDDTAVYYCARSPYGHYAMDYWGQGTTVTVSSASTKGPSVFPLAPSSKSTSGGTAALGCLVKDYFPEPVTVSWNSGALTSGVHTFPAVLQSSGLYSLSSVVTVPSSSLGTQTYICNVNHKPSNTKVDKKVEPKSCDKTHTCPPCPAPELLGGPSVFLFPPKPKDTLMISRTPEVTCVVVDVSHEDPEVKFNWYVDGVEVHNAKTKPREEQYNSTYRVVSVLTVLHQDWLNGKEYKCKVSNKALPAPIEKTISKAKGQPREPQVYTLPPSREEMTKNQVSLTCLVKGFYPSDIAVEWESNGQPENNYKTTPPVLDSDGSFFLYSKLTVDKSRWQQGNVFSCSVMHEALHNHYTQKSLSLSPGK
atgaaacacctgtggttcttcctcctgctggtggcagctcccagatgggtgctgagcgaagtgcagctggttcagtctggcgccgaagtgaaaaagcctggcgcctctgtgaaggtgtcctgcaaggccagcggctacagcttcaccgactacaacatgtactgggtccgacaggcccctggccagtctcttgagtggatgggctacatcgacccctacaacggcgacaccacctacaaccagaaattccagggcagagtgaccatgaccagagacaccagcatcagcaccgcctacatggaactgagccggctgagatccgatgacaccgccgtgtactactgcgccagatctccttacggccactacgccatggattactggggccagggcaccacagtgacagttagctcagcctccaccaagggcccaagcgtcttccccctggcaccctcctccaagagcacctctggcggcacagccgccctgggctgcctggtcaaggactacttccccgaacccgtgaccgtgagctggaactcaggcgccctgaccagcggcgtgcacaccttccccgctgtcctgcagtcctcaggactctactccctcagcagcgtggtgaccgtgccctccagcagcttgggcacccagacctacatctgcaacgtgaatcacaagcccagcaacaccaaggtggacaagaaggttgagcccaaatcttgtgacaaaactcacacatgcccaccctgcccagcacctgaactcctggggggaccctcagtcttcctcttccccccaaaacccaaggacaccctcatgatctcccggacccctgaggtcacatgcgtggtggtggacgtgagccacgaagaccctgaggtcaagttcaactggtacgtggacggcgtggaggtgcataatgccaagacaaagccccgggaggagcagtacaacagcacgtaccgggtggtcagcgtcctcaccgtcctgcaccaggactggctgaatggcaaggagtacaagtgcaaggtctccaacaaagccctcccagcccccatcgagaaaaccatctccaaagccaaaggccagccccgggaaccacaggtgtacaccctgcccccatcccgggaggagatgaccaagaaccaggtcagcctgacctgcctggtcaaaggcttctatcccagcgacatcgccgtggagtgggagagcaatggccagcccgagaacaactacaagaccacccctcccgtgctggactccgacggctccttcttcctctacagcaagctcaccgtggacaagagcaggtggcagcagggcaacgtcttctcatgctccgtgatgcatgaggctctgcacaaccactacacccagaagagcctctccctgtctcccggcaaa

SEQ ID NO: 6 - protein, 468 aa, synthetic construct
  REGION 1..468: note = Synthetic Construct
MKHLWFFLLLVAAPRWVLSEVQLVQSGAEVKKPGASVKVSCKASGYSFTDYNMYWVRQAPGQSLEWMGYIDPYNGDTTYNQKFQGRVTMTRDTSISTAYMELSRLRSDDTAVYYCARSPYGHYAMDYWGQGTTVTVSSASTKGPSVFPLAPSSKSTSGGTAALGCLVKDYFPEPVTVSWNSGALTSGVHTFPAVLQSSGLYSLSSVVTVPSSSLGTQTYICNVNHKPSNTKVDKKVEPKSCDKTHTCPPCPAPELLGGPSVFLFPPKPKDTLMISRTPEVTCVVVDVSHEDPEVKFNWYVDGVEVHNAKTKPREEQYNSTYRVVSVLTVLHQDWLNGKEYKCKVSNKALPAPIEKTISKAKGQPREPQVYTLPPSREEMTKNQVSLTCLVKGFYPSDIAVEWESNGQPENNYKTTPPVLDSDGSFFLYSKLTVDKSRWQQGNVFSCSVMHEALHNHYTQKSLSLSPGK

SEQ ID NO: 7 - DNA, 1404 bp, synthetic construct
  misc_feature 1..1404: note = nucleotide sequence coding hmAb-H551 heavy chain
  source 1..1404: mol_type = other DNA
  CDS 1..>1404: protein_id = 8; translation = MKHLWFFLLLVAAPRWVLSEVQLVQSGAEVKKPGASVKVSCKASGYSFTDYNMYWVRQAPGQSLEWMGYIDPYNGDTTYNQKFQGRVTMTRDTSSSTAYMELSRLRSDDTAVYYCARSPYGHYAMDYWGQGTTVTVSSASTKGPSVFPLAPSSKSTSGGTAALGCLVKDYFPEPVTVSWNSGALTSGVHTFPAVLQSSGLYSLSSVVTVPSSSLGTQTYICNVNHKPSNTKVDKKVEPKSCDKTHTCPPCPAPELLGGPSVFLFPPKPKDTLMISRTPEVTCVVVDVSHEDPEVKFNWYVDGVEVHNAKTKPREEQYNSTYRVVSVLTVLHQDWLNGKEYKCKVSNKALPAPIEKTISKAKGQPREPQVYTLPPSREEMTKNQVSLTCLVKGFYPSDIAVEWESNGQPENNYKTTPPVLDSDGSFFLYSKLTVDKSRWQQGNVFSCSVMHEALHNHYTQKSLSLSPGK
atgaaacacctgtggttcttcctcctgctggtggcagctcccagatgggtgctgagcgaagtgcagctggttcagtctggcgccgaagtgaaaaagcctggcgcctctgtgaaggtgtcctgcaaggccagcggctacagcttcaccgactacaacatgtactgggtccgacaggcccctggccagtctcttgagtggatgggctacatcgacccctacaacggcgacaccacctacaaccagaaattccagggcagagtgaccatgaccagagacaccagcagcagcaccgcctacatggaactgagcagactgagaagcgacgacaccgccgtgtactactgcgccagatctccttacggccactacgccatggattactggggccagggcaccacagtgacagttagctcagcctccaccaagggcccaagcgtcttccccctggcaccctcctccaagagcacctctggcggcacagccgccctgggctgcctggtcaaggactacttccccgaacccgtgaccgtgagctggaactcaggcgccctgaccagcggcgtgcacaccttccccgctgtcctgcagtcctcaggactctactccctcagcagcgtggtgaccgtgccctccagcagcttgggcacccagacctacatctgcaacgtgaatcacaagcccagcaacaccaaggtggacaagaaggttgagcccaaatcttgtgacaaaactcacacatgcccaccctgcccagcacctgaactcctggggggaccctcagtcttcctcttccccccaaaacccaaggacaccctcatgatctcccggacccctgaggtcacatgcgtggtggtggacgtgagccacgaagaccctgaggtcaagttcaactggtacgtggacggcgtggaggtgcataatgccaagacaaagccccgggaggagcagtacaacagcacgtaccgggtggtcagcgtcctcaccgtcctgcaccaggactggctgaatggcaaggagtacaagtgcaaggtctccaacaaagccctcccagcccccatcgagaaaaccatctccaaagccaaaggccagccccgggaaccacaggtgtacaccctgcccccatcccgggaggagatgaccaagaaccaggtcagcctgacctgcctggtcaaaggcttctatcccagcgacatcgccgtggagtgggagagcaatggccagcccgagaacaactacaagaccacccctcccgtgctggactccgacggctccttcttcctctacagcaagctcaccgtggacaagagcaggtggcagcagggcaacgtcttctcatgctccgtgatgcatgaggctctgcacaaccactacacccagaagagcctctccctgtctcccggcaaa

SEQ ID NO: 8 - protein, 468 aa, synthetic construct
  REGION 1..468: note = Synthetic Construct
MKHLWFFLLLVAAPRWVLSEVQLVQSGAEVKKPGASVKVSCKASGYSFTDYNMYWVRQAPGQSLEWMGYIDPYNGDTTYNQKFQGRVTMTRDTSSSTAYMELSRLRSDDTAVYYCARSPYGHYAMDYWGQGTTVTVSSASTKGPSVFPLAPSSKSTSGGTAALGCLVKDYFPEPVTVSWNSGALTSGVHTFPAVLQSSGLYSLSSVVTVPSSSLGTQTYICNVNHKPSNTKVDKKVEPKSCDKTHTCPPCPAPELLGGPSVFLFPPKPKDTLMISRTPEVTCVVVDVSHEDPEVKFNWYVDGVEVHNAKTKPREEQYNSTYRVVSVLTVLHQDWLNGKEYKCKVSNKALPAPIEKTISKAKGQPREPQVYTLPPSREEMTKNQVSLTCLVKGFYPSDIAVEWESNGQPENNYKTTPPVLDSDGSFFLYSKLTVDKSRWQQGNVFSCSVMHEALHNHYTQKSLSLSPGK

SEQ ID NO: 9 - DNA, 1404 bp, synthetic construct
  misc_feature 1..1404: note = nucleotide sequence coding hmAb-H11a heavy chain
  source 1..1404: mol_type = other DNA
  CDS 1..>1404: protein_id = 10; translation = MKHLWFFLLLVAAPRWVLSEVQLVQSGAEVKKPGASVKVSCKASGYSFTDYNMYWVRQAPGQSLEWMGYIDPYNGDTTYNQKFQGRVTITADKSKSTAYMELSSLRSEDTAVYYCARSPYGHYAMDYWGQGTLVTVSSASTKGPSVFPLAPSSKSTSGGTAALGCLVKDYFPEPVTVSWNSGALTSGVHTFPAVLQSSGLYSLSSVVTVPSSSLGTQTYICNVNHKPSNTKVDKKVEPKSCDKTHTCPPCPAPELLGGPSVFLFPPKPKDTLMISRTPEVTCVVVDVSHEDPEVKFNWYVDGVEVHNAKTKPREEQYNSTYRVVSVLTVLHQDWLNGKEYKCKVSNKALPAPIEKTISKAKGQPREPQVYTLPPSREEMTKNQVSLTCLVKGFYPSDIAVEWESNGQPENNYKTTPPVLDSDGSFFLYSKLTVDKSRWQQGNVFSCSVMHEALHNHYTQKSLSLSPGK
atgaaacacctgtggttcttcctcctgctggtggcagctcccagatgggtgctgagcgaagtgcagctggttcagtctggcgccgaagtgaaaaagcctggcgcctctgtgaaggtgtcctgcaaggccagcggctacagcttcaccgactacaacatgtactgggtccgacaggcccctggccagtctcttgagtggatgggctacatcgacccctacaacggcgacaccacctacaaccagaaattccagggcagagtgaccatcaccgccgacaagagcaagagcaccgcctacatggaactgagcagcctgagaagcgaggacaccgccgtgtactactgcgccagatctccttacggccactacgccatggattactggggccagggcacactggttaccgttagctcagcctccaccaagggcccaagcgtcttccccctggcaccctcctccaagagcacctctggcggcacagccgccctgggctgcctggtcaaggactacttccccgaacccgtgaccgtgagctggaactcaggcgccctgaccagcggcgtgcacaccttccccgctgtcctgcagtcctcaggactctactccctcagcagcgtggtgaccgtgccctccagcagcttgggcacccagacctacatctgcaacgtgaatcacaagcccagcaacaccaaggtggacaagaaggttgagcccaaatcttgtgacaaaactcacacatgcccaccctgcccagcacctgaactcctggggggaccctcagtcttcctcttccccccaaaacccaaggacaccctcatgatctcccggacccctgaggtcacatgcgtggtggtggacgtgagccacgaagaccctgaggtcaagttcaactggtacgtggacggcgtggaggtgcataatgccaagacaaagccccgggaggagcagtacaacagcacgtaccgggtggtcagcgtcctcaccgtcctgcaccaggactggctgaatggcaaggagtacaagtgcaaggtctccaacaaagccctcccagcccccatcgagaaaaccatctccaaagccaaaggccagccccgggaaccacaggtgtacaccctgcccccatcccgggaggagatgaccaagaaccaggtcagcctgacctgcctggtcaaaggcttctatcccagcgacatcgccgtggagtgggagagcaatggccagcccgagaacaactacaagaccacccctcccgtgctggactccgacggctccttcttcctctacagcaagctcaccgtggacaagagcaggtggcagcagggcaacgtcttctcatgctccgtgatgcatgaggctctgcacaaccactacacccagaagagcctctccctgtctcccggcaaa

SEQ ID NO: 10 - protein, 468 aa, synthetic construct
  REGION 1..468: note = Synthetic Construct
MKHLWFFLLLVAAPRWVLSEVQLVQSGAEVKKPGASVKVSCKASGYSFTDYNMYWVRQAPGQSLEWMGYIDPYNGDTTYNQKFQGRVTITADKSKSTAYMELSSLRSEDTAVYYCARSPYGHYAMDYWGQGTLVTVSSASTKGPSVFPLAPSSKSTSGGTAALGCLVKDYFPEPVTVSWNSGALTSGVHTFPAVLQSSGLYSLSSVVTVPSSSLGTQTYICNVNHKPSNTKVDKKVEPKSCDKTHTCPPCPAPELLGGPSVFLFPPKPKDTLMISRTPEVTCVVVDVSHEDPEVKFNWYVDGVEVHNAKTKPREEQYNSTYRVVSVLTVLHQDWLNGKEYKCKVSNKALPAPIEKTISKAKGQPREPQVYTLPPSREEMTKNQVSLTCLVKGFYPSDIAVEWESNGQPENNYKTTPPVLDSDGSFFLYSKLTVDKSRWQQGNVFSCSVMHEALHNHYTQKSLSLSPGK

SEQ ID NO: 11 - DNA, 449 bp, synthetic construct
  misc_feature 1..449: note = nucleotide fragment comprising nucleotide sequences coding humanlight chain signal sequence and human kappa light chain constantregion
  source 1..449: mol_type = other DNA
gcctccggactctagagccaccatggtgctgcagacccaggtgttcatctccctgctgctgtggatctccggcgcgtacggcgatatcgtgatgattaaacgtacggtggccgccccctccgtgttcatcttccccccctccgacgagcagctgaagtccggcaccgcctccgtggtgtgcctgctgaataacttctaccccagagaggccaaggtgcagtggaaggtggacaacgccctgcagtccgggaactcccaggagagcgtgaccgagcaggacagcaaggacagcacctacagcctgagcagcaccctgaccctgagcaaagccgactacgagaagcacaaggtgtacgcctgcgaggtgacccaccagggcctgagctcccccgtcaccaagagcttcaacaggggggagtgttaggggcccgtttaaacgggggaggcta

SEQ ID NO: 12 - DNA, 366 bp, synthetic construct
  misc_feature 1..366: note = nucleotide sequence coding variable region of hmAb-L11 lightchain
  source 1..366: mol_type = other DNA
ctgtggatctccggcgcgtacggcgatatccagatgacacagagccctagcagcctgtctgccagcgtgggagacagagtgaccatcacatgcaaggccagccaggatgtgtccaccgccgtggattggtatcagcagaagcctggcaaggcccctaagctgctgatcaactgggccagcacaagacacacaggcgtgcccagcagattttctggcagcggctctggcaccgacttcaccctgaccatatctagcctgcagcctgaggacttcgccacctactactgcagacagcactacagcacccctttcacctttggccagggcaccaaggtggaaatcaagcgtacggtggccgccccctcc

SEQ ID NO: 13 - DNA, 1117 bp, synthetic construct
  misc_feature 1..1117: note = nucleotide fragment comprising nucleotide sequences coding humanheavy chain signal sequence and human G1 heavy chain constantregion
  source 1..1117: mol_type = other DNA
gggtctagagccaccatgaaacacctgtggttcttcctcctgctggtggcagctcccagatgggtgctgagccaggtgcaattgtgcaggcggttagctcagcctccaccaagggcccaagcgtcttccccctggcaccctcctccaagagcacctctggcggcacagccgccctgggctgcctggtcaaggactacttccccgaacccgtgaccgtgagctggaactcaggcgccctgaccagcggcgtgcacaccttccccgctgtcctgcagtcctcaggactctactccctcagcagcgtggtgaccgtgccctccagcagcttgggcacccagacctacatctgcaacgtgaatcacaagcccagcaacaccaaggtggacaagaaggttgagcccaaatcttgtgacaaaactcacacatgcccaccctgcccagcacctgaactcctggggggaccctcagtcttcctcttccccccaaaacccaaggacaccctcatgatctcccggacccctgaggtcacatgcgtggtggtggacgtgagccacgaagaccctgaggtcaagttcaactggtacgtggacggcgtggaggtgcataatgccaagacaaagccccgggaggagcagtacaacagcacgtaccgggtggtcagcgtcctcaccgtcctgcaccaggactggctgaatggcaaggagtacaagtgcaaggtctccaacaaagccctcccagcccccatcgagaaaaccatctccaaagccaaaggccagccccgggaaccacaggtgtacaccctgcccccatcccgggaggagatgaccaagaaccaggtcagcctgacctgcctggtcaaaggcttctatcccagcgacatcgccgtggagtgggagagcaatggccagcccgagaacaactacaagaccacccctcccgtgctggactccgacggctccttcttcctctacagcaagctcaccgtggacaagagcaggtggcagcagggcaacgtcttctcatgctccgtgatgcatgaggctctgcacaaccactacacccagaagagcctctccctgtctcccggcaaatgagatatcgggcccgtttaaacggg

SEQ ID NO: 14 - DNA, 396 bp, synthetic construct
  misc_feature 1..396: note = nucleotide sequence coding variable region of hmAb-H11 heavychain
  source 1..396: mol_type = other DNA
agctcccagatgggtgctgagcgaagttcagctggttcagtctggcgccgaagtgaagaaacctggcgcctctgtgaaggtgtcctgcaaggccagcggctacagcttcaccgactacaacatgtactgggtccgacaggcccctggccagtctcttgagtggatgggctacatcgacccctacaacggcgacaccacctacaaccagaaattccagggcagagtgaccatcaccgccgacacctctacaagcaccgcctacatggaactgagcagcctgagaagcgaggacaccgccgtgtactactgcgccagatctccttacggccactacgccatggattactggggccagggaaccctggtcacagttagctcagcctccaccaagggccc

SEQ ID NO: 15 - DNA, 396 bp, synthetic construct
  misc_feature 1..396: note = nucleotide sequence coding variable region of hmAb-H541 heavychain
  source 1..396: mol_type = other DNA
agctcccagatgggtgctgagcgaagtgcagctggttcagtctggcgccgaagtgaaaaagcctggcgcctctgtgaaggtgtcctgcaaggccagcggctacagcttcaccgactacaacatgtactgggtccgacaggcccctggccagtctcttgagtggatgggctacatcgacccctacaacggcgacaccacctacaaccagaaattccagggcagagtgaccatgaccagagacaccagcatcagcaccgcctacatggaactgagccggctgagatccgatgacaccgccgtgtactactgcgccagatctccttacggccactacgccatggattactggggccagggcaccacagtgacagttagctcagcctccaccaagggccc

SEQ ID NO: 16 - DNA, 396 bp, synthetic construct
  misc_feature 1..396: note = nucleotide sequence coding variable region of hmAb-H551 heavychain
  source 1..396: mol_type = other DNA
agctcccagatgggtgctgagcgaagtgcagctggttcagtctggcgccgaagtgaaaaagcctggcgcctctgtgaaggtgtcctgcaaggccagcggctacagcttcaccgactacaacatgtactgggtccgacaggcccctggccagtctcttgagtggatgggctacatcgacccctacaacggcgacaccacctacaaccagaaattccagggcagagtgaccatgaccagagacaccagcagcagcaccgcctacatggaactgagcagactgagaagcgacgacaccgccgtgtactactgcgccagatctccttacggccactacgccatggattactggggccagggcaccacagtgacagttagctcagcctccaccaagggccc

SEQ ID NO: 17 - DNA, 396 bp, synthetic construct
  misc_feature 1..396: note = nucleotide sequence coding variable region of hmAb-H11a heavychain
  source 1..396: mol_type = other DNA
agctcccagatgggtgctgagcgaagtgcagctggttcagtctggcgccgaagtgaaaaagcctggcgcctctgtgaaggtgtcctgcaaggccagcggctacagcttcaccgactacaacatgtactgggtccgacaggcccctggccagtctcttgagtggatgggctacatcgacccctacaacggcgacaccacctacaaccagaaattccagggcagagtgaccatcaccgccgacaagagcaagagcaccgcctacatggaactgagcagcctgagaagcgaggacaccgccgtgtactactgcgccagatctccttacggccactacgccatggattactggggccagggcacactggttaccgttagctcagcctccaccaagggccc

SEQ ID NO: 18 - protein, 281 aa, Homo sapiens
MSAQESCLSLIKYFLFVFNLFFFVLGSLIFCFGIWILIDKTSFVSFVGLAFVPLQIWSKVLAISGIFTMGIALLGCVGALKELRCLLGLYFGMLLLLFATQITLGILISTQRAQLERSLRDVVEKTIQKYGTNPEETAAEESWDYVQFQLRCCGWHYPQDWFQVLILRGNGSEAHRVPCSCYNLSATNDSTILDKVILPQLSRLGHLARSRHSADICAVPAESHIYREGCAQGLQKWLHNNLISIVGICLGVGLLELGFMTLSIFLCRNLDHVYNRLARYR

SEQ ID NO: 19 - protein, 11 aa, synthetic construct
  REGION 1..11: note = CDRL1 sequence of humanized anti-CD37 antibody
KASQDVSTAVD

SEQ ID NO: 20 - protein, 7 aa, synthetic construct
  REGION 1..7: note = CDRL2 sequence of humanized anti-CD37 antibody
WASTRHT

SEQ ID NO: 21 - protein, 9 aa, synthetic construct
  REGION 1..9: note = CDRL3 sequence of humanized anti-CD37 antibody
RQHYSTPFT

SEQ ID NO: 22 - protein, 10 aa, synthetic construct
  REGION 1..10: note = CDRH1 sequence of humanized anti-CD37 antibody
GYSFTDYNMY

SEQ ID NO: 23 - protein, 10 aa, synthetic construct
  REGION 1..10: note = CDRH2 sequence of humanized anti-CD37 antibody
YIDPYNGDTT

SEQ ID NO: 24 - protein, 10 aa, synthetic construct
  REGION 1..10: note = CDRH3 sequence of humanized anti-CD37 antibody
SPYGHYAMDY